European Patent Application EP 4 768 589 A1, published July 1, 2026. Title: Novel promoter and uses thereof. Applicant: CJ CheilJedang Corporation. The sequence listing filed with the application follows.

SEQUENCE LISTING (43 sequences)

SEQ ID NO: 1 - DNA, 86 bp, synthetic construct
  misc_feature 1..86: note = Po2 (wild type)
  source 1..86: mol_type = other DNA
caataatcgtgaattttggcagcaacagaattatgtggtataatggaaacgtgcaaaagcatagattattggaggagatcaaaaca

SEQ ID NO: 2 - DNA, 41 bp, synthetic construct
  misc_feature 1..41: note = primer
  source 1..41: mol_type = other DNA
ctctagaactagtggatccccccaataatcgtgaattttgg

SEQ ID NO: 3 - DNA, 44 bp, synthetic construct
  misc_feature 1..44: note = primer
  source 1..44: mol_type = other DNA
aaagttcttctcctttactcattgttttgatctcctccaataat

SEQ ID NO: 4 - DNA, 47 bp, synthetic construct
  misc_feature 1..47: note = primer
  source 1..47: mol_type = other DNA
aaagttcttctcctttactcatatgtgttttgatctcctccaataat

SEQ ID NO: 5 - DNA, 50 bp, synthetic construct
  misc_feature 1..50: note = primer
  source 1..50: mol_type = other DNA
aaagttcttctcctttactcatactatgtgttttgatctcctccaataat

SEQ ID NO: 6 - DNA, 44 bp, synthetic construct
  misc_feature 1..44: note = primer
  source 1..44: mol_type = other DNA
attattggaggagatcaaaacaatgagtaaaggagaagaacttt

SEQ ID NO: 7 - DNA, 44 bp, synthetic construct
  misc_feature 1..44: note = primer
  source 1..44: mol_type = other DNA
tgatatcgaattcctgcagcccttatttgtagagctcatccatg

SEQ ID NO: 8 - DNA, 47 bp, synthetic construct
  misc_feature 1..47: note = primer
  source 1..47: mol_type = other DNA
attattggaggagatcaaaacacatatgagtaaaggagaagaacttt

SEQ ID NO: 9 - DNA, 50 bp, synthetic construct
  misc_feature 1..50: note = primer
  source 1..50: mol_type = other DNA
attattggaggagatcaaaacaactagtatgagtaaaggagaagaacttt

SEQ ID NO: 10 - DNA, 25 bp, synthetic construct
  misc_feature 1..25: note = primer
  source 1..25: mol_type = other DNA
gggctgcaggaattcgatatcaagc

SEQ ID NO: 11 - DNA, 25 bp, synthetic construct
  misc_feature 1..25: note = primer
  source 1..25: mol_type = other DNA
gggggatccactagttctagagcgg

SEQ ID NO: 12 - DNA, 39 bp, synthetic construct
  misc_feature 1..39: note = primer
  source 1..39: mol_type = other DNA
gaaaaattttttatcttatccaataatcgtgaattttgg

SEQ ID NO: 13 - DNA, 40 bp, synthetic construct
  misc_feature 1..40: note = primer
  source 1..40: mol_type = other DNA
agttcttctcctttactcattgttttgatctcctccaata

SEQ ID NO: 14 - DNA, 40 bp, synthetic construct
  misc_feature 1..40: note = primer
  source 1..40: mol_type = other DNA
tattggaggagatcaaaacaatgagtaaaggagaagaact

SEQ ID NO: 15 - DNA, 40 bp, synthetic construct
  misc_feature 1..40: note = primer
  source 1..40: mol_type = other DNA
aggcgggctgccccggggacttatttgtagagctcatcca

SEQ ID NO: 16 - DNA, 20 bp, synthetic construct
  misc_feature 1..20: note = primer
  source 1..20: mol_type = other DNA
gtccccggggcagcccgcct

SEQ ID NO: 17 - DNA, 20 bp, synthetic construct
  misc_feature 1..20: note = primer
  source 1..20: mol_type = other DNA
gataagataaaaaatttttc

SEQ ID NO: 18 - DNA, 40 bp, synthetic construct
  misc_feature 1..40: note = primer
  source 1..40: mol_type = other DNA
aatgtagtgaggtggatgcaatgagtaaaggagaagaact

SEQ ID NO: 19 - DNA, 40 bp, synthetic construct
  misc_feature 1..40: note = primer
  source 1..40: mol_type = other DNA
gaaaaattttttatcttatcatgagtaaaggagaagaact

SEQ ID NO: 20 - DNA, 40 bp, synthetic construct; identical to SEQ ID NO: 18
  misc_feature 1..40: note = primer
  source 1..40: mol_type = other DNA

SEQ ID NO: 21 - DNA, 3423 bp, synthetic construct
  misc_feature 1..3423: note = pyc gene encoding Pyruvate Carboxylase derived from Corynebacterium glutamicum (Ncgl0659)
  source 1..3423: mol_type = other DNA
gtgtcgactcacacatcttcaacgcttccagcattcaaaaagatcttggtagcaaaccgcggcgaaatcgcggtccgtgctttccgtgcagcactcgaaaccggtgcagccacggtagctatttacccccgtgaagatcggggatcattccaccgctcttttgcttctgaagctgtccgcattggtaccgaaggctcaccagtcaaggcgtacctggacatcgatgaaattatcggtgcagctaaaaaagttaaagcagatgccatttacccgggatacggcttcctgtctgaaaatgcccagcttgcccgcgagtgtgcggaaaacggcattacttttattggcccaaccccagaggttcttgatctcaccggtgataagtctcgcgcggtaaccgccgcgaagaaggctggtctgccagttttggcggaatccaccccgagcaaaaacatcgatgagatcgttaaaagcgctgaaggccagacttaccccatctttgtgaaggcagttgccggtggtggcggacgcggtatgcgttttgttgcttcacctgatgagcttcgcaaattagcaacagaagcatctcgtgaagctgaagcggctttcggcgatggcgcggtatatgtcgaacgtgctgtgattaaccctcagcatattgaagtgcagatccttggcgatcacactggagaagttgtacacctttatgaacgtgactgctcactgcagcgtcgtcaccaaaaagttgtcgaaattgcgccagcacagcatttggatccagaactgcgtgatcgcatttgtgcggatgcagtaaagttctgccgctccattggttaccagggcgcgggaaccgtggaattcttggtcgatgaaaagggcaaccacgtcttcatcgaaatgaacccacgtatccaggttgagcacaccgtgactgaagaagtcaccgaggtggacctggtgaaggcgcagatgcgcttggctgctggtgcaaccttgaaggaattgggtctgacccaagataagatcaagacccacggtgcagcactgcagtgccgcatcaccacggaagatccaaacaacggcttccgcccagataccggaactatcaccgcgtaccgctcaccaggcggagctggcgttcgtcttgacggtgcagctcagctcggtggcgaaatcaccgcacactttgactccatgctggtgaaaatgacctgccgtggttccgactttgaaactgctgttgctcgtgcacagcgcgcgttggctgagttcaccgtgtctggtgttgcaaccaacattggtttcttgcgtgcgttgctgcgggaagaggacttcacttccaagcgcatcgccaccggattcattgccgatcacccgcacctccttcaggctccacctgctgatgatgagcagggacgcatcctggattacttggcagatgtcaccgtgaacaagcctcatggtgtgcgtccaaaggatgttgcagctcctatcgataagctgcctaacatcaaggatctgccactgccacgcggttcccgtgaccgcctgaagcagcttggcccagccgcgtttgctcgtgatctccgtgagcaggacgcactggcagttactgataccaccttccgcgatgcacaccagtctttgcttgcgacccgagtccgctcattcgcactgaagcctgcggcagaggccgtcgcaaagctgactcctgagcttttgtccgtggaggcctggggcggcgcgacctacgatgtggcgatgcgtttcctctttgaggatccgtgggacaggctcgacgagctgcgcgaggcgatgccgaatgtaaacattcagatgctgcttcgcggccgcaacaccgtgggatacaccccgtacccagactccgtctgccgcgcgtttgttaaggaagctgccagctccggcgtggacatcttccgcatcttcgacgcgcttaacgacgtctcccagatgcgtccagcaatcgacgcagtcctggagaccaacaccgcggtagccgaggtggctatggcttattctggtgatctctctgatccaaatgaaaagctctacaccctggattactacctaaagatggcagaggagatcgtcaagtctggcgctcacatcttggccattaaggatatggctggtctgcttcgcccagctgcggtaaccaagctggtcaccgcactgcgccgtgaattcgatctgccagtgcacgtgcacacccacgacactgcgggtggccagctggcaacctactttgctgcagctcaagctggtgcagatgctgttgacggtgcttccgcaccactgtctggcaccacctcccagccatccctgtctgccattgttgctgcattcgcgcacacccgtcgcgataccggtttgagcctcgaggctgtttctgacctcgagccgtactgggaagcagtgcgcggactgtacctgccatttgagtctggaaccccaggcccaaccggtcgcgtctaccgccacgaaatcccaggcggacagttgtccaacctgcgtgcacaggccaccgcactgggccttgcggatcgtttcgaactcatcgaagacaactacgcagccgttaatgagatgctgggacgcccaaccaaggtcaccccatcctccaaggttgttggcgacctcgcactccacctcgttggtgcgggtgtggatccagcagactttgctgccgatccacaaaagtacgacatcccagactctgtcatcgcgttcctgcgcggcgagcttggtaaccctccaggtggctggccagagccactgcgcacccgcgcactggaaggccgctccgaaggcaaggcacctctgacggaagttcctgaggaagagcaggcgcacctcgacgctgatgattccaaggaacgtcgcaatagcctcaaccgcctgctgttcccgaagccaaccgaagagttcctcgagcaccgtcgccgcttcggcaacacctctgcgctggatgatcgtgaattcttctacggcctggtcgaaggccgcgagactttgatccgcctgccagatgtgcgcaccccactgcttgttcgcctggatgcgatctctgagccagacgataagggtatgcgcaatgttgtggccaacgtcaacggccagatccgcccaatgcgtgtgcgtgaccgctccgttgagtctgtcaccgcaaccgcagaaaaggcagattcctccaacaagggccatgttgctgcaccattcgctggtgttgtcaccgtgactgttgctgaaggtgatgaggtcaaggctggagatgcagtcgcaatcatcgaggctatgaagatggaagcaacaatcactgcttctgttgacggcaaaatcgatcgcgttgtggttcctgctgcaacgaaggtggaaggtggcgacttgatcgtcgtcgtttcctaa

SEQ ID NO: 22 - DNA, 34 bp, synthetic construct
  misc_feature 1..34: note = primer
  source 1..34: mol_type = other DNA
aagtttagaaatattcaataatcgtgaattttgg

SEQ ID NO: 23 - DNA, 32 bp, synthetic construct
  misc_feature 1..32: note = primer
  source 1..32: mol_type = other DNA
gatgtgtgagtcgacactgttttgatctcctc

SEQ ID NO: 24 - DNA, 26 bp, synthetic construct
  misc_feature 1..26: note = primer
  source 1..26: mol_type = other DNA
agctcggtacccgagccccatccgtt

SEQ ID NO: 25 - DNA, 27 bp, synthetic construct
  misc_feature 1..27: note = primer
  source 1..27: mol_type = other DNA
tcacgattattgaatatttctaaactt

SEQ ID NO: 26 - DNA, 28 bp, synthetic construct
  misc_feature 1..28: note = primer
  source 1..28: mol_type = other DNA
atcaaaacagtgtcgactcacacatctt

SEQ ID NO: 27 - DNA, 30 bp, synthetic construct
  misc_feature 1..30: note = primer
  source 1..30: mol_type = other DNA
actctagaggatccccacaaagatggggta

SEQ ID NO: 28 - DNA, 1134 bp, synthetic construct
  misc_feature 1..1134: note = metX gene encoding Homoserine O-acetyltransferase derived from Corynebacterium glutamicum (Ncgl0624)
  source 1..1134: mol_type = other DNA
atgcccaccctcgcgccttcaggtcaacttgaaatccaagcgatcggtgatgtctccaccgaagccggagcaatcattacaaacgctgaaatcgcctatcaccgctggggtgaataccgcgtagataaagaaggacgcagcaatgtcgttctcatcgaacacgccctcactggagattccaacgcagccgattggtgggctgacttgctcggtcccggcaaagccatcaacactgatatttactgcgtgatctgtaccaacgtcatcggtggttgcaacggttccaccggacctggctccatgcatccagatggaaatttctggggtaatcgcttccccgccacgtccattcgtgatcaggtaaacgccgaaaaacaattcctcgacgcactcggcatcaccacggtcgccgcagtacttggtggttccatgggtggtgcccgcaccctagagtgggccgcaatgtacccagaaactgttggcgcagctgctgttcttgcagtttctgcacgcgccagcgcctggcaaatcggcattcaatccgcccaaattaaggcgattgaaaacgaccaccactggcacgaaggcaactactacgaatccggctgcaacccagccaccggactcggcgccgcccgacgcatcgcccacctcacctaccgtggcgaactagaaatcgacgaacgcttcggcaccaaagcccaaaagaacgaaaacccactcggtccctaccgcaagcccgaccagcgcttcgccgtggaatcctacttggactaccaagcagacaagctagtacagcgtttcgacgccggctcctacgtcttgctcaccgacgccctcaaccgccacgacattggtcgcgaccgcggaggcctcaacaaggcactcgaatccatcaaagttccagtccttgtcgcaggcgtagataccgatattttgtacccctaccaccagcaagaacacctctccagaaacctgggaaatctactggcaatggcaaaaatcgtatcccctgtcggccacgatgctttcctcaccgaaagccgccaaatggatcgcatcgtgaggaacttcttcagcctcatctccccagacgaagacaacccttcgacctacatcgagttctacatctaa

SEQ ID NO: 29 - DNA, 44 bp, synthetic construct
  misc_feature 1..44: note = primer
  source 1..44: mol_type = other DNA
ctgaaggcgcgagggtgggcattgttttgatctcctccaataat

SEQ ID NO: 30 - DNA, 44 bp, synthetic construct
  misc_feature 1..44: note = primer
  source 1..44: mol_type = other DNA
attattggaggagatcaaaacaatgcccaccctcgcgccttcag

SEQ ID NO: 31 - DNA, 44 bp, synthetic construct
  misc_feature 1..44: note = primer
  source 1..44: mol_type = other DNA
tgatatcgaattcctgcagcccttagatgtagaactcgatgtag

SEQ ID NO: 32 - DNA, 1104 bp, synthetic construct
  misc_feature 1..1104: note = ilvE gene encoding branched-chain-amino-acid transaminase derived from Corynebacterium glutamicum (Ncgl2123)
  source 1..1104: mol_type = other DNA
atgacgtcattagagttcacagtaacccgtaccgaaaatccgacgtcacccgatcgtctgaaggaaattcttgccgcaccgaagttcggtaagtacttcaccgaccacatggtgaccattgactggaacgagtcggaaggctggcacaacgcccaattagtgccatacgcgccgattcctatggatcctgccaccaccgtattccactacggacaggcaatttttgagggaattaaggcctaccgccattcggacgaaaccatcaagactttccgtcctgatgaaaacgccgagcgtatgcagcgttcagcagctcgaatggcaatgccacagttgccaaccgaggactttattaaagcacttgaactgctggtagacgcggatcaggattgggttcctgagtacggcggggaagcttccctctacctgcgcccattcatgatctccaccgaaattggcttgggtgtcagcccagctgatgcctacaagttcctggtcatcgcatccccagtcggcgcttacttcaccggtggaatcaagcctgtttccgtctggctgagcgaagattacgtccgcgctgcacccggcggaactggtgacgccaaatttgctggcaactacgcggcttctttgcttgcccagtcccaggctgcggaaaagggctgtgaccaggtcgtatggttggatgccatcgagcacaagtacatcgaagaaatgggtggcatgaaccttgggttcatctaccgcaacggcgaccacgtcaagctagtcacccctgaactttccggctcactacttccaggcatcactcgcaagtcacttctacaagtagcacgcgacttgggctacgaagtagaagagcgaaagatcaccaccaccgagtgggaagaagacgcaaagtctggcgccatgaccgaggcatttgcttgcggtactgcagctgttatcacccctgttggcaccgtgaaatcagctcacggcaccttcgaagtgaacaacaatgaagtcggagaaatcacgatgaagcttcgtgaaaccctcaccggaattcagcaaggaaacgttgaagaccaaaacggatggctttacccactggttggctaa

SEQ ID NO: 33 - DNA, 33 bp, synthetic construct
  misc_feature 1..33: note = primer
  source 1..33: mol_type = other DNA
tcatcccataaaatcaataatcgtgaattttgg

SEQ ID NO: 34 - DNA, 28 bp, synthetic construct
  misc_feature 1..28: note = primer
  source 1..28: mol_type = other DNA
taatgacgtcattgttttgatctcctcc

SEQ ID NO: 35 - DNA, 30 bp, synthetic construct
  misc_feature 1..30: note = primer
  source 1..30: mol_type = other DNA
ttcgagctcggtacccccgtgccggaagcg

SEQ ID NO: 36 - DNA, 32 bp, synthetic construct
  misc_feature 1..32: note = primer
  source 1..32: mol_type = other DNA
ttcacgattattgattttatgggatgaatagc

SEQ ID NO: 37 - DNA, 31 bp, synthetic construct
  misc_feature 1..31: note = primer
  source 1..31: mol_type = other DNA
ggagatcaaaacaatgacgtcattagagttc

SEQ ID NO: 38 - DNA, 29 bp, synthetic construct
  misc_feature 1..29: note = primer
  source 1..29: mol_type = other DNA
tctagaggatccccatgaccaggaacttg

SEQ ID NO: 39 - DNA, 86 bp, synthetic construct
  misc_feature 1..86: note = Po2.1 (21A>C)
  source 1..86: mol_type = other DNA
caataatcgtgaattttggccgcaacagaattatgtggtataatggaaacgtgcaaaagcatagattattggaggagatcaaaaca

SEQ ID NO: 40 - DNA, 86 bp, synthetic construct
  misc_feature 1..86: note = Po2.2 (19G>A)
  source 1..86: mol_type = other DNA
caataatcgtgaattttgacagcaacagaattatgtggtataatggaaacgtgcaaaagcatagattattggaggagatcaaaaca

SEQ ID NO: 41 - DNA, 89 bp, synthetic construct
  misc_feature 1..89: note = Po2.3 (added "cat" at 3' end)
  source 1..89: mol_type = other DNA
caataatcgtgaattttggcagcaacagaattatgtggtataatggaaacgtgcaaaagcatagattattggaggagatcaaaacacat

SEQ ID NO: 42 - DNA, 92 bp, synthetic construct
  misc_feature 1..92: note = Po2.4 (added "actagt" at 3' end)
  source 1..92: mol_type = other DNA
caataatcgtgaattttggcagcaacagaattatgtggtataatggaaacgtgcaaaagcatagattattggaggagatcaaaacaactagt

SEQ ID NO: 43 - DNA, 5802 bp, synthetic construct
  misc_feature 1..5802: note = pDC24
  source 1..5802: mol_type = other DNA
gttcgcttgctgtccataaaaccgcccagtctagctatcgccatgtaagcccactgcaagctacctgctttctctttgcgcttgcgttttcccttgtccagatagcccagtagctgacattcatccggggtcagcaccgtttctgcggactggctttctacgtgttccgcttcctttagcagcccttgcgccctgagtgcttgcggcagcgtgaagctagcttttatcgccattcgccattcaggctgcgcaactgttgggaagggcgatcggtgcgggcctcttcgctattacgccagctggcgaaagggggatgtgctgcaaggcgattaagttgggtaacgccagggttttcccagtcacgacgttgtaaaacgacggccagtgaattcgagctcggtacccggggatcctctagagtcgacctgcaggcatgcaagcttggcgtaatcatggtcatagctgtttcctgtgtgaaattgttatccgctcacaattccacacaacatacgagccggaagcataaagtgtaaagcctggggtgcctaatgagtgagctaactcacattaattgcgttgcgctcactgcccgctttccagtcgggaaacctgtcgtgccagctgcattaatgaatcggccaacgcgcggggagaggcggtttgcgtattgggcgctcttccgcttcctcgctcactgactcgctgcgctcggtcgttcggctgcggcgagcggtatcagctcactcaaaggcggtaatacggttatccacagaatcaggggataacgcaggaaagaacatgtgagcaaaaggccagcaaaaggccaggaaccgtaaaaaggccgcgttgctggcgtttttccataggctccgcccccctgacgagcatcacaaaaatcgacgctcaagtcagaggtggcgaaacccgacaggactataaagataccaggcgtttccccctggaagctccctcgtgcgctctcctgttccgaccctgccgcttaccggatacctgtccgcctttctcccttcgggaagcgtggcgctttctcaatgctcacgctgtaggtatctcagttcggtgtaggtcgttcgctccaagctgggctgtgtgcacgaaccccccgttcagcccgaccgctgcgccttatccggtaactatcgtcttgagtccaacccggtaagacacgacttatcgccactggcagcagccactggtaacaggattagcagagcgaggtatgtaggcggtgctacagagttcttgaagtggtggcctaactacggctacactagaaggacagtatttggtatctgcgctctgctgaagccagttaccttcggaaaaagagttggtagctcttgatccggcaaacaaaccaccgctggtagcggtggtttttttgtttgcaagcagcagattacgcgcagaaaaaaaggatctcaagaagatcctttgatcttttctacggggtctgacgctcagtggaacgaaaactcacgttaagggattttggtcatgagattatcaaaaaggatcttcacctagatccttttggggtgggcgaagaactccagcatgagatccccgcgctggaggatcatccagccctgatagaaacagaagccactggagcacctcaaaaacaccatcatacactaaatcagtaagttggcagcatcacccgacgcactttgcgccgaataaatacctgtgacggaagatcacttcgcagaataaataaatcctggtgtccctgttgataccgggaagccctgggccaacttttggcgaaaatgagacgttgatcggcacgtaagaggttccaactttcaccataatgaaataagatcactaccgggcgtattttttgagttatcgagattttcaggagctgatagaaacagaagccactggagcacctcaaaaacaccatcatacactaaatcagtaagttggcagcatcacccgacgcactttgcgccgaataaatacctgtgacggaagatcacttcgcagaataaataaatcctggtgtccctgttgataccgggaagccctgggccaacttttggcgaaaatgagacgttgatcggcacgtaagaggttccaactttcaccataatgaaataagatcactaccgggcgtattttttgagttatcgagattttcaggagctctttggcatcgtctctcgcctgtcccctcagttcagtaatttcctgcatttgcctgtttccagtcggtagatattccacaaaacagcagggaagcagcgcttttccgctgcataaccctgcttcggggtcattatagcgattttttcggtatatccatcctttttcgcacgatatacaggattttgccaaagggttcgtgtagactttccttggtgtatccaacggcgtcagccgggcaggataggtgaagtaggcccacccgcgagcgggtgttccttcttcactgtcccttattcgcacctggcggtgctcaacgggaatcctgctctgcgaggctggccggctaccgccggcgtaacagatgagggcaagcggatggctgatgaaaccaagccaaccaggaagggcagcccacctatcaaggtgtactgccttccagacgaacgaagagcgattgaggaaaaggcggcggcggccggcatgagcctgtcggcctacctgctggccgtcggccagggctacaaaatcacgggcgtcgtggactatgagcacgtccgcgagggcgtcccggaaaacgattccgaagcccaacctttcatagaaggcggcggtggaatcgaaatctcgtgatggcaggttgggcgtcgcttggtcggtcatttcgaaaaaggttaggaatacggttagccatttgcctgcttttatatagttcatatgggattcacctttatgttgataagaaataaaagaaaatgccaataggatatcggcattttcttttgcgtttttatttgttaactgttaattgtccttgttcaaggatgctgtctttgacaacagatgttttcttgcctttgatgttcagcaggaagctcggcgcaaacgttgattgtttgtctgcgtagaatcctctgtttgtcatatagcttgtaatcacgacattgtttcctttcgcttgaggtacagcgaagtgtgagtaagtaaaggttacatcgttaggcggatcaagatccatttttaacacaaggccagttttgttcagcggcttgtatgggccagttaaagaattagaaacataaccaagcatgtaaatatcgttagacgtaatgccgtcaatcgtcatttttgatccgcgggagtcagtgaacaggtaccatttgccgttcattttaaagacgttcgcgcgttcaatttcatctgttactgtgttagatgcaatcagcggtttcatcacttttttcagtgtgtaatcatcgtttagctcaatcataccgagagcgccgtttgctaactcagccgtgcgttttttatcgctttgcagaagtttttgactttcttgacggaagaatgatgtgcttttgccatagtatgctttgttaaataaagattcttcgccttggtagccatcttcagttccagtgtttgcttcaaatactaagtatttgtggcctttatcttctacgtagtgaggatctctcagcgtatggttgtcgcctgagctgtagttgccttcatcgatgaactgctgtacattttgatacgtttttccgtcaccgtcaaagattgatttataatcctctacaccgttgatgttcaaagagctgtctgatgctgatacgttaacttgtgcagttgtcagtgtttgtttgccgtaatgtttaccggagaaatcagtgtagaataaacggatttttccgtcagatgtaaatgtggctgaacctgaccattcttgtgtttggtcttttaggatagaatcatttgcatcgaatttgtcgctgtctttaaagacgcggccagcgtttttccagctgtcaatagaagtttcgccgactttttgatagaacatgtaaatcgatgtgtcatccgcatttttaggatctccggctaatgcaaagacgatgtggtagccgtgatagtttgcgacagtgccgtcagcgttttgtaatggccagctgtcccaaacgtccaggccttttgcagaagagatatttttaattgtggacgaatcaaattcagaaacttgatatttttcatttttttgctgttcagggatttgcagcatatcatggcgtgtaatatgggaaatgccgtatgtttccttatatggcttttggttcgtttctttcgcaaacgcttgagttgcgcctcctgccagcagtgcggtagtaaaggttaatactgttgcttgttttgcaaactttttgatgttcatcgttcatgtctccttttttatgtactgtgttagcggtctgcttcttccagccctcctgtttgaagatggcaagttagttacgcacaataaaaaaagacctaaaatatgtaaggggtgacgccaaagtatacactttgccctttacacattttaggtcttgcctgctttatcagtaacaaacccgcgcgatttacttttcgacctcattctattagactctcgtttggattgcaactggtctattttcctcttttgtttgatagaaaatcataaaaggatttgcagactacgggcctaaagaactaaaaaatctatctgtttcttttcattctctgtattttttatagtttctgttgcatgggcataaagttgcctttttaatcacaattcagaaaatatcataatatctcatttcactaaataatagtgaacggcaggtatatgtgatgggttaaaaaggatcaccccagagtcccgctcagaagaactcgtcaagaaggcgatagaaggcgatgcgctgcgaatcgggagcggcgataccgtaaagcacgaggaagcggtcagcccattcgccgccaagctcttcagcaatatcacgggtagccaacgctatgtcctgatagcggtccgccacacccagccggccacagtcgatgaatccagaaaagcggccattttccaccatgatattcggcaagcaggcatcgccatgggtcacgacgagatcctcgccgtcgggcatccgcgccttgagcctggcgaacagttcggctggcgcgagcccctgatgctcttcgtccagatcatcctgatcgacaagaccggcttccatccgagtacgtgctcgctcgatgcgatgtttcgcttggtggtcgaatgggcaggtagccggatcaagcgtatgcagccgccgcattgcatcagccatgatggatactttctcggcaggagcaaggtgagatgacaggagatcctgccccggcacttcgcccaatagcagccagtcccttcccgcttcagtgacaacgtcgagacagctgcgcaaggaacgcccgtcgtggccagccacgatagccgcgctgcctcgtcttggagttcattcagggcaccggacaggtcggtcttgacaaaaagaaccgggcgcccctgcgctgacagccggaacacggcggcatcagagcagccgattgtctgttgtgcccagtcatagccgaatagcctctccacccaagcggccggagaacctgcgtgcaatccatcttgttcaatcatgcgaaacgatcctcatcctgtctcttgatcagatcttgatcccctgcgccatcagatccttggcggcaagaaagccatccagtttactttgcagggcttcccaaccttaccagagggcgccccagctggcaattccg